European Patent Application EP 4 549 575 A1, published May 7, 2025. Title: ANTIMICROBIAL PEPTIDES FOR THE CONTAINMENT OF OOMYCETES IN AGRICULTURE. Applicant: Universita degli Studi di Milano. Application EP. The sequence listing filed with the application follows.

SEQUENCE LISTING (41 sequences)

SEQ ID NO: 1 - protein, 9 aa, synthetic construct
  REGION 1..9: note = Antimicrobial cyclic peptide CP20
  MOD_RES 1: note = X is B-alanine
XRWMLVYRR

SEQ ID NO: 2 - protein, 9 aa, synthetic construct
  REGION 1..9: note = Antimicrobial cyclic peptide CP32
  MOD_RES 1: note = X is B Ala
XGRLRWLRV

SEQ ID NO: 3 - protein, 9 aa, synthetic construct
  REGION 1..9: note = Antimicrobial linear peptide LP20
  MOD_RES 1: note = X is Ac-B Ala
XRWMLVYRR

SEQ ID NO: 4 - protein, 9 aa, synthetic construct
  REGION 1..9: note = Antimicrobial linear peptide LP32
  MOD_RES 1: note = X is Ac-B Ala
XGRLRWLRV

SEQ ID NO: 5 - DNA, 24 bp, synthetic construct
  misc_feature 1..24: note = Nucleotide sequence encoding for CP20/LP20 peptide
  misc_feature 1: note = M is A or C
  misc_feature 3: note = N is A, C, G or T
  misc_feature 10: note = Y is C or T
  misc_feature 12: note = N is A, C, G or T
  misc_feature 15: note = N is A, C, G or T
  misc_feature 18: note = Y is C or T
  misc_feature 19: note = M is A or C
  misc_feature 21: note = N is A, C, G or T
  misc_feature 2: note = M is A or C
  misc_feature 24: note = N is A, C, G or T
  source 1..24: mol_type = other DNA
mgntggatgytngtntaymgnmgn

SEQ ID NO: 6 - DNA, 24 bp, synthetic construct
  misc_feature 1..24: note = Nucleotide sequence encoding for CP32/LP32 peptide
  misc_feature 3: note = N is A, C, G or T
  misc_feature 4: note = M is A or C
  misc_feature 6: note = N is A, C, G or T
  misc_feature 7: note = Y is C or T
  misc_feature 9: note = N is A, C, G or T
  misc_feature 10: note = M is A or C
  misc_feature 12: note = N is A, C, G or T
  misc_feature 16: note = Y is C or T
  misc_feature 18: note = N is A, C, G or T
  misc_feature 19: note = M is A or C
  misc_feature 21: note = N is A, C, G or T
  misc_feature 24: note = N is A, C, G or T
  source 1..24: mol_type = other DNA
ggnmgnytnmgntggytnmgngtn

SEQ ID NO: 7 - protein, 9 aa, synthetic construct
  REGION 1..9: note = Peptidomimetic variant of CP20 peptide
  MOD_RES 1: note = X is B Ala
  MOD_RES 5: note = Z is aza-Leu
XRWMZVYRR

SEQ ID NO: 8 - protein, 9 aa, synthetic construct
  REGION 1..9: note = Peptidomimetic variant of CP20 peptide
  MOD_RES 1: note = X is B Ala
  MOD_RES 5: note = Z is hydrazino Leu
XRWMZVYRR

SEQ ID NO: 9 - protein, 9 aa, synthetic construct
  REGION 1..9: note = Peptidomimetic variant of CP20 peptide
  MOD_RES 1: note = X is B Ala
  MOD_RES 4: note = Z is CF3 Met
XRWZLVYRR

SEQ ID NO: 10 - protein, 9 aa, synthetic construct
  REGION 1..9: note = Peptidomimetic variant of CP20 peptide
  MOD_RES 1: note = X is B Ala
  MOD_RES 2: note = N is (D) R where D is D amino acid
  MOD_RES 3: note = N is (D) Trp where D is D amino acid
  MOD_RES 7: note = N is (D) Tyr where D is D amino acid
  MOD_RES 9: note = N is (D) Arg where D is D amino acid
XNNMLVNRN

SEQ ID NO: 11 - protein, 9 aa, synthetic construct
  REGION 1..9: note = Peptidomimetic variant of CP20 peptide
  MOD_RES 1: note = X is B Ala
  MOD_RES 2: note = N is (D) Arg where D means D amino acid
  MOD_RES 3: note = N is (D) Trp where D means D amino acid
  MOD_RES 7: note = N is (D) Tyr where D means D amino acid
XNNMLVNRR

SEQ ID NO: 12 - protein, 9 aa, synthetic construct
  REGION 1..9: note = Peptidomimetic variant of CP20 peptide
  MOD_RES 1: note = X is B ala
  MOD_RES 3: note = N is (D)W where D is D aminoacid
  MOD_RES 7: note = Z is (D)Y where D is D aminoacid
XRNMLVZRR

SEQ ID NO: 13 - protein, 9 aa, synthetic construct
  REGION 1..9: note = Peptidomimetic variant of CP20 peptide
  MOD_RES 1: note = X is B-Ala
  MOD_RES 5: note = Z is hydrazino Leu
XRWAZVYRR

SEQ ID NO: 14 - protein, 9 aa, synthetic construct
  REGION 1..9: note = Peptidomimetic variant of CP20 peptide
  MOD_RES 1: note = X is B-Ala
  MOD_RES 3: note = N is D(W) wherein D is D aminoacid
  MOD_RES 7: note = Z is D(Y) wherein D is D aminoacid
XRNMLVZRR

SEQ ID NO: 15 - protein, 9 aa, synthetic construct
  REGION 1..9: note = Peptidomimetic variant of CP32 peptide
  MOD_RES 1: note = X is B-Ala
  MOD_RES 5: note = N is D(R) wherein D is D aminoacid
  MOD_RES 6: note = Z is D(W) wherein D is D aminoacid
XGRLNZLRV

SEQ ID NO: 16 - protein, 9 aa, synthetic construct
  REGION 1..9: note = Peptidomimetic variant of CP32 peptide
  MOD_RES 1: note = X is B-Ala
  MOD_RES 5: note = N is D(R) wherein D is D aminoacid
  MOD_RES 7: note = Z is D(L) wherein D is D aminoacid
XGRLNWZRV

SEQ ID NO: 17 - protein, 9 aa, synthetic construct
  REGION 1..9: note = Peptidomimetic variant of CP32 peptide
  MOD_RES 1: note = X is B-Ala
  MOD_RES 3: note = N is D(R) wherein D is D aminoacid
  MOD_RES 5: note = Z is D(R) wherein D is D aminoacid
  MOD_RES 6: note = N is D(W) wherein D is D aminoacid
XGNLZNLRV

SEQ ID NO: 18 - protein, 9 aa, synthetic construct
  REGION 1..9: note = Peptidomimetic variant of CP32 peptide
  MOD_RES 1: note = X is B-Ala
  MOD_RES 6: note = N is D(W) wherein D is D aminoacid
  MOD_RES 7: note = Z is D(L) wherein D is D aminoacid
XGRLRNZRV

SEQ ID NO: 19 - protein, 9 aa, synthetic construct
  REGION 1..9: note = Peptidomimetic variant of CP32 peptide
  MOD_RES 1: note = X is B-Ala
  MOD_RES 6: note = N is D(W) wherein D is D aminoacid
  MOD_RES 8: note = Z is D(R) wherein D is D aminoacid
XGRLRNLZV

SEQ ID NO: 20 - protein, 9 aa, synthetic construct
  REGION 1..9: note = Peptidomimetic variant of CP32 peptide
  MOD_RES 1: note = X is B-Ala
  MOD_RES 3: note = N is D(R) wherein D is D aminoacid
  MOD_RES 6: note = Z is D(W) wherein D is D aminoacid
XGNLRZLRV

SEQ ID NO: 21 - protein, 9 aa, synthetic construct
  REGION 1..9: note = Peptidomimetic variant of CP32 peptide
  MOD_RES 1: note = X is B-Ala
  MOD_RES 6: note = N is azahomo Trp
XGRLRNLRV

SEQ ID NO: 22 - protein, 9 aa, synthetic construct
  REGION 1..9: note = Peptidomimetic variant of CP32 peptide
  MOD_RES 1: note = X is B-Ala
  MOD_RES 7: note = N is aza Leu
XGRLRWNRV

SEQ ID NO: 23 - protein, 9 aa, synthetic construct
  REGION 1..9: note = Peptidomimetic variant of CP32 peptide
  MOD_RES 1: note = X is B-Ala
  MOD_RES 6: note = N is hydrazino Trp
XGRLRNLRV

SEQ ID NO: 24 - protein, 9 aa, synthetic construct
  REGION 1..9: note = Peptidomimetic variant of CP32 peptide
  MOD_RES 1: note = X is B-Ala
  MOD_RES 7: note = N is hydrazino Leu
XGRLRWNRV

SEQ ID NO: 25 - protein, 9 aa, synthetic construct
  REGION 1..9: note = Peptidomimetic variant of CP32 peptide
  MOD_RES 1: note = X is B-Ala
  MOD_RES 4: note = N is hydrazino Leu
XGRNRWLRV

SEQ ID NO: 26 - protein, 9 aa, synthetic construct
  REGION 1..9: note = Met-Ala version of CP20
  MOD_RES 1: note = X is B Ala
XRWALVYRR

SEQ ID NO: 27 - protein, 9 aa, synthetic construct
  REGION 1..9: note = LP20 Ala2 variant
  MOD_RES 1: note = X is Ac-B Ala
XAWMLVYRR

SEQ ID NO: 28 - protein, 9 aa, synthetic construct
  REGION 1..9: note = LP20 Ala3 variant
  MOD_RES 1: note = X is Ac-B Ala
XRAMLVYRR

SEQ ID NO: 29 - protein, 9 aa, synthetic construct
  REGION 1..9: note = LP20 Ala5 variant
  MOD_RES 1: note = X is Ac-B Ala
XRWMAVYRR

SEQ ID NO: 30 - protein, 9 aa, synthetic construct
  REGION 1..9: note = LP20 Ala6 variant
  MOD_RES 1: note = X is Ac-B Ala
XRWMLAYRR

SEQ ID NO: 31 - protein, 9 aa, synthetic construct
  REGION 1..9: note = LP20 Ala7 variant
  MOD_RES 1: note = X is Ac-B Ala
XRWMLVARR

SEQ ID NO: 32 - protein, 9 aa, synthetic construct
  REGION 1..9: note = LP20 Ala8 variant
  MOD_RES 1: note = X is Ac-B Ala
XRWMLVYAR

SEQ ID NO: 33 - protein, 9 aa, synthetic construct
  REGION 1..9: note = LP20 Ala9 variant
  MOD_RES 1: note = X is Ac-B Ala
XRWMLVYRA

SEQ ID NO: 34 - protein, 9 aa, synthetic construct
  REGION 1..9: note = LP32 Ala2 variant
  MOD_RES 1: note = X is Ac-B Ala
XARLRWLRV

SEQ ID NO: 35 - protein, 9 aa, synthetic construct
  REGION 1..9: note = LP32 Ala3 peptide variant
  MOD_RES 1: note = X is B Ala
XGALRWLRV

SEQ ID NO: 36 - protein, 9 aa, synthetic construct
  REGION 1..9: note = LP32 Ala4
  MOD_RES 1: note = X is Ac-B Ala
XGRARWLRV

SEQ ID NO: 37 - protein, 9 aa, synthetic construct
  REGION 1..9: note = LP32 Ala5 variant
  MOD_RES 1: note = X is Ac-B Ala
XGRLAWLRV

SEQ ID NO: 38 - protein, 9 aa, synthetic construct
  REGION 1..9: note = LP32 Ala6 variant
  MOD_RES 1: note = X is Ac-B Ala
XGRLRALRV

SEQ ID NO: 39 - protein, 9 aa, synthetic construct
  REGION 1..9: note = LP32 Ala7 variant
  MOD_RES 1: note = X is Ac-B Ala
XGRLRWARV

SEQ ID NO: 40 - protein, 9 aa, synthetic construct
  REGION 1..9: note = LP32 Ala8 variant
  MOD_RES 1: note = X is Ac-B Ala
XGRLRWLAV

SEQ ID NO: 41 - protein, 9 aa, synthetic construct
  REGION 1..9: note = LP32 Ala9 variant
  MOD_RES 1: note = X is Ac-B Ala
XGRLRWLRA